European Patent Specification EP 3 883 591 B1, published November 13, 2024. Title: Relaxin Receptor 1 for use in Treatament and Prevention of Heart Failure. Applicant: Universität Heidelberg. The sequence listing filed with the application follows.

SEQUENCE LISTING (38 sequences)

SEQ ID NO: 1 - DNA, 2301 bp, Artificial
  codon-optimized human RXFP1 coding sequence
atggactacaaggacgacgatgacaagatgacatctggttctgtcttcttctacatcttaatttttggaaaatatttttctcatgggggtggacaggatgtcaagtgctcccttggctatttcccctgtgggaacatcacaaagtgcttgcctcagctcctgcactgtaacggtgtggacgactgcgggaatcaggccgatgaggacaactgtggagacaacaatggatggtctctgcaatttgacaaatattttgccagttactacaaaatgacttcccaatatccttttgaggcagaaacacctgaatgtttggtcggttctgtgccagtgcaatgtctttgccaaggtctggagcttgactgtgatgaaaccaatttacgagctgttccatcggtttcttcaaatgtgactgcaatgtcacttcagtggaacttaataagaaaacttcctcctgattgcttcaagaattatcatgatcttcagaagctgtacctgcaaaacaataagattacatccatctccatctatgctttcagaggactgaatagccttactaaactgtatctcagtcataacagaataaccttcctgaagccgggtgtttttgaagatcttcacagactagaatggctgataattgaagataatcacctcagtcgaatttccccaccaacattttatggactaaattctcttattctcttagtcctgatgaataacgtcctcacccgtttacctgataaacctctctgtcaacacatgccaagactacattggctggaccttgaaggcaaccatatccataatttaagaaatttgacttttatttcctgtagtaatttaactgttttagtgatgaggaaaaacaaaattaatcacttaaatgaaaatacttttgcacctctccagaaactggatgaattggatttaggaagtaataagattgaaaatcttccaccgcttatattcaaggacctgaaggagctgtcacaattgaatctttcctataatccaatccagaaaattcaagcaaaccaatttgattatcttgtcaaactcaagtctctcagcctagaagggattgaaatttcaaatatccaacaaaggatgtttagacctcttatgaatctctctcacatatattttaagaaattccagtactgtgggtatgcaccacatgttcgcagctgtaaaccaaacactgatggaatttcatctctagagaatctcttggcaagcattattcagagagtatttgtctgggttgtatctgctgttacctgctttggaaacatttttgtcatttgcatgcgaccttatatcaggtctgagaacaagctgtatgccatgtcaatcatttctctctgctgtgccgactgcttaatgggaatatatttattcgtgatcggaggctttgacctaaagtttcgtggagaatacaataagcatgcgcagctgtggatggagagtactcattgtcagcttgtaggatctttggccattctgtccacagaagtatcagttttactgttaacatttctgacattggaaaaatacatctgcattgtctatccttttagatgtgtgagacctggaaaatgcagaacaattacagttctgattctcatttggattactggttttatagtggctttcattccattgagcaataaggaatttttcaaaaactactatggcaccaatggagtatgcttccctcttcattcagaagatacagaaagtattggagcccagatttattcagtggcaatttttcttggtattaatttggccgcatttatcatcatagttttttcctatggaagcatgttttatagtgttcatcaaagtgccataacagcaactgaaatacggaatcaagttaaaaaagagatgatccttgccaaacgttttttctttatagtatttactgatgcattatgctggatacccatttttgtagtgaaatttctttcactgcttcaggtagaaataccaggtaccataacctcttgggtagtgatttttattctgcccattaacagtgctttgaacccaattctctatactctgaccacaagaccatttaaagaaatgattcatcggttttggtataactacagacaaagaaaatctatggacagcaaaggtcagaaaacatatgctccatcattcatctgggtggaaatgtggccactccaggagatgccacctgagttaatgaagccggaccttttcacatacccctgtgaaatgtcactgatttctcaatcaacgagactcaattcctattcatga

SEQ ID NO: 2 - protein, 766 aa, Homo sapiens
MDYKDDDDKMTSGSVFFYILIFGKYFSHGGGQDVKCSLGYFPCGNITKCLPQLLHCNGVDDCGNQADEDNCGDNNGWSLQFDKYFASYYKMTSQYPFEAETPECLVGSVPVQCLCQGLELDCDETNLRAVPSVSSNVTAMSLQWNLIRKLPPDCFKNYHDLQKLYLQNNKITSISIYAFRGLNSLTKLYLSHNRITFLKPGVFEDLHRLEWLIIEDNHLSRISPPTFYGLNSLILLVLMNNVLTRLPDKPLCQHMPRLHWLDLEGNHIHNLRNLTFISCSNLTVLVMRKNKINHLNENTFAPLQKLDELDLGSNKIENLPPLIFKDLKELSQLNLSYNPIQKIQANQFDYLVKLKSLSLEGIEISNIQQRMFRPLMNLSHIYFKKFQYCGYAPHVRSCKPNTDGISSLENLLASIIQRVFVWVVSAVTCFGNIFVICMRPYIRSENKLYAMSIISLCCADCLMGIYLFVIGGFDLKFRGEYNKHAQLWMESTHCQLVGSLAILSTEVSVLLLTFLTLEKYICIVYPFRCVRPGKCRTITVLILIWITGFIVAFIPLSNKEFFKNYYGTNGVCFPLHSEDTESIGAQIYSVAIFLGINLAAFIIIVFSYGSMFYSVHQSAITATEIRNQVKKEMILAKRFFFIVFTDALCWIPIFVVKFLSLLQVEIPGTITSWVVIFILPINSALNPILYTLTTRPFKEMIHRFWYNYRQRKSMDSKGQKTYAPSFIWVEMWPLQEMPPELMKPDLFTYPCEMSLISQSTRLNSYS

SEQ ID NO: 3 - DNA, 2274 bp, Artificial
  5' shortened codon-optimized human RXFP1 coding sequence
atgacatctggttctgtcttcttctacatcttaatttttggaaaatatttttctcatgggggtggacaggatgtcaagtgctcccttggctatttcccctgtgggaacatcacaaagtgcttgcctcagctcctgcactgtaacggtgtggacgactgcgggaatcaggccgatgaggacaactgtggagacaacaatggatggtctctgcaatttgacaaatattttgccagttactacaaaatgacttcccaatatccttttgaggcagaaacacctgaatgtttggtcggttctgtgccagtgcaatgtctttgccaaggtctggagcttgactgtgatgaaaccaatttacgagctgttccatcggtttcttcaaatgtgactgcaatgtcacttcagtggaacttaataagaaagcttcctcctgattgcttcaagaattatcatgatcttcagaagctgtacctgcaaaacaataagattacatccatctccatctatgctttcagaggactgaatagccttactaaactgtatctcagtcataacagaataaccttcctgaagccgggtgtttttgaagatcttcacagactagaatggctgataattgaagataatcacctcagtcgaatttccccaccaacattttatggactaaattctcttattctcttagtcctgatgaataacgtcctcacccgtttacctgataaacctctctgtcaacacatgccaagactacattggctggaccttgaaggcaaccatatccataatttaagaaatttgacttttatttcctgcagtaatttaactgttttagtgatgaggaaaaacaaaattaatcacttaaatgaaaatacttttgcacctctccagaaactggatgaattggatttaggaagtaataagattgaaaatcttccaccgcttatattcaaggacctgaaggagctgtcacaattgaatctttcctataatccaatccagaaaattcaagcaaaccaatttgattatcttgtcaaactcaagtctctcagcctagaagggattgaaatttcaaatatccaacaaaggatgtttagacctcttatgaatctctctcacatatattttaagaaattccagtactgtgggtatgcaccacatgttcgcagctgtaaaccaaacactgatggaatttcatctctagagaatctcttggcaagcattattcagagagtatttgtctgggttgtatctgcagttacctgctttggaaacatttttgtcatttgcatgcgaccttatatcaggtctgagaacaagctgtatgccatgtcaatcatttctctctgctgtgccgactgcttaatgggaatatatttattcgtgatcggaggctttgacctaaagtttcgtggagaatacaataagcatgcgcagctgtggatggagagtactcattgtcagcttgtaggatctttggccattctgtccacagaagtatcagttttactgttaacatttctgacattggaaaaatacatctgcattgtctatccttttagatgtgtgagacctggaaaatgcagaacaattacagttctgattctcatttggattactggttttatagtggctttcattccattgagcaataaggaatttttcaaaaactactatggcaccaatggagtatgcttccctcttcattcagaagatacagaaagtattggagcccagatttattcagtggcaatttttcttggtattaatttggccgcatttatcatcatagttttttcctatggaagcatgttttatagtgttcatcaaagtgccataacagcaactgaaatacggaatcaagttaaaaaagagatgatccttgccaaacgttttttctttatagtatttactgatgcattatgctggatacccatttttgtagtgaaatttctttcactgcttcaggtagaaataccaggtaccataacctcttgggtagtgatttttattctgcccattaacagtgctttgaacccaattctctatactctgaccacaagaccatttaaagaaatgattcatcggttttggtataactacagacaaagaaaatctatggacagcaaaggtcagaaaacatatgctccatcattcatctgggtggaaatgtggccactgcaggagatgccacctgagttaatgaagccggaccttttcacatacccctgtgaaatgtcactgatttctcaatcaacgagactcaattcctattcatga

SEQ ID NO: 4 - protein, 757 aa, Homo sapiens
MTSGSVFFYILIFGKYFSHGGGQDVKCSLGYFPCGNITKCLPQLLHCNGVDDCGNQADEDNCGDNNGWSLQFDKYFASYYKMTSQYPFEAETPECLVGSVPVQCLCQGLELDCDETNLRAVPSVSSNVTAMSLQWNLIRKLPPDCFKNYHDLQKLYLQNNKITSISIYAFRGLNSLTKLYLSHNRITFLKPGVFEDLHRLEWLIIEDNHLSRISPPTFYGLNSLILLVLMNNVLTRLPDKPLCQHMPRLHWLDLEGNHIHNLRNLTFISCSNLTVLVMRKNKINHLNENTFAPLQKLDELDLGSNKIENLPPLIFKDLKELSQLNLSYNPIQKIQANQFDYLVKLKSLSLEGIEISNIQQRMFRPLMNLSHIYFKKFQYCGYAPHVRSCKPNTDGISSLENLLASIIQRVFVWVVSAVTCFGNIFVICMRPYIRSENKLYAMSIISLCCADCLMGIYLFVIGGFDLKFRGEYNKHAQLWMESTHCQLVGSLAILSTEVSVLLLTFLTLEKYICIVYPFRCVRPGKCRTITVLILIWITGFIVAFIPLSNKEFFKNYYGTNGVCFPLHSEDTESIGAQIYSVAIFLGINLAAFIIIVFSYGSMFYSVHQSAITATEIRNQVKKEMILAKRFFFIVFTDALCWIPIFVVKFLSLLQVEIPGTITSWVVIFILPINSALNPILYTLTTRPFKEMIHRFWYNYRQRKSMDSKGQKTYAPSFIWVEMWPLQEMPPELMKPDLFTYPCEMSLISQSTRLNSYS

SEQ ID NO: 5 - DNA, 2274 bp, Homo sapiens; identical to SEQ ID NO: 3

SEQ ID NO: 6 - DNA, 518 bp, Artificial
  CMV enhancer
actagttattaatagtaatcaattacggggtcattagttcatagcccatatatggagttccgcgttacataacttacggtaaatggcccgcctggctgaccgcccaacgacccccgcccattgacgtcaataatgacgtatgttcccatagtaacgccaatagggactttccattgacgtcaatgggtggagtatttacggtaaactgcccacttggcagtacatcaagtgtatcatatgccaagtacgccccctattgacgtcaatgacggtaaatggcccgcctggcattatgcccagtacatgaccttatgggactttcctacttggcagtacatctacgtattagtcatcgctattaccatggtgatgcggttttggcagtacatcaatgggcgtggatagcggtttgactcacggggatttccaagtctccaccccattgacgtcaatgggagtttgttttggcaccaaaatcaacgggactttccaaaatgtcgtaacactccgccccatgc

SEQ ID NO: 7 - DNA, 263 bp, Artificial
  MLC260 promoter
gacccagagcacagagcatcgttcccaggccaggccccagccactgtctctttaaccttgaaggcatttttgggtctcacgtgtccacccaggcgggtgtcggactttgaacggctcttacttcagaagaacggcatggggtgggggggcttaggtggcctctgcctcacctacaactgccaaaagtggtcatggggttatttttaaccccagggaagaggtatttattgttccacagcaggggccggccagcaggctccttg

SEQ ID NO: 8 - DNA, 3112 bp, Artificial
  CMV-MLC260 -Modified Human RXFP1
actagttattaatagtaatcaattacggggtcattagttcatagcccatatatggagttccgcgttacataacttacggtaaatggcccgcctggctgaccgcccaacgacccccgcccattgacgtcaataatgacgtatgttcccatagtaacgccaatagggactttccattgacgtcaatgggtggagtatttacggtaaactgcccacttggcagtacatcaagtgtatcatatgccaagtacgccccctattgacgtcaatgacggtaaatggcccgcctggcattatgcccagtacatgaccttatgggactttcctacttggcagtacatctacgtattagtcatcgctattaccatggtgatgcggttttggcagtacatcaatgggcgtggatagcggtttgactcacggggatttccaagtctccaccccattgacgtcaatgggagtttgttttggcaccaaaatcaacgggactttccaaaatgtcgtaacactccgccccatgcggccgctctaggacccagagcacagagcatcgttcccaggccaggccccagccactgtctctttaaccttgaaggcatttttgggtctcacgtgtccacccaggcgggtgtcggactttgaacggctcttacttcagaagaacggcatggggtgggggggcttaggtggcctctgcctcacctacaactgccaaaagtggtcatggggttatttttaaccccagggaagaggtatttattgttccacagcaggggccggccagcaggctccttgaattctgcagaccatggactacaaggacgacgatgacaagatgacatctggttctgtcttcttctacatcttaatttttggaaaatatttttctcatgggggtggacaggatgtcaagtgctcccttggctatttcccctgtgggaacatcacaaagtgcttgcctcagctcctgcactgtaacggtgtggacgactgcgggaatcaggccgatgaggacaactgtggagacaacaatggatggtctctgcaatttgacaaatattttgccagttactacaaaatgacttcccaatatccttttgaggcagaaacacctgaatgtttggtcggttctgtgccagtgcaatgtctttgccaaggtctggagcttgactgtgatgaaaccaatttacgagctgttccatcggtttcttcaaatgtgactgcaatgtcacttcagtggaacttaataagaaaacttcctcctgattgcttcaagaattatcatgatcttcagaagctgtacctgcaaaacaataagattacatccatctccatctatgctttcagaggactgaatagccttactaaactgtatctcagtcataacagaataaccttcctgaagccgggtgtttttgaagatcttcacagactagaatggctgataattgaagataatcacctcagtcgaatttccccaccaacattttatggactaaattctcttattctcttagtcctgatgaataacgtcctcacccgtttacctgataaacctctctgtcaacacatgccaagactacattggctggaccttgaaggcaaccatatccataatttaagaaatttgacttttatttcctgtagtaatttaactgttttagtgatgaggaaaaacaaaattaatcacttaaatgaaaatacttttgcacctctccagaaactggatgaattggatttaggaagtaataagattgaaaatcttccaccgcttatattcaaggacctgaaggagctgtcacaattgaatctttcctataatccaatccagaaaattcaagcaaaccaatttgattatcttgtcaaactcaagtctctcagcctagaagggattgaaatttcaaatatccaacaaaggatgtttagacctcttatgaatctctctcacatatattttaagaaattccagtactgtgggtatgcaccacatgttcgcagctgtaaaccaaacactgatggaatttcatctctagagaatctcttggcaagcattattcagagagtatttgtctgggttgtatctgctgttacctgctttggaaacatttttgtcatttgcatgcgaccttatatcaggtctgagaacaagctgtatgccatgtcaatcatttctctctgctgtgccgactgcttaatgggaatatatttattcgtgatcggaggctttgacctaaagtttcgtggagaatacaataagcatgcgcagctgtggatggagagtactcattgtcagcttgtaggatctttggccattctgtccacagaagtatcagttttactgttaacatttctgacattggaaaaatacatctgcattgtctatccttttagatgtgtgagacctggaaaatgcagaacaattacagttctgattctcatttggattactggttttatagtggctttcattccattgagcaataaggaatttttcaaaaactactatggcaccaatggagtatgcttccctcttcattcagaagatacagaaagtattggagcccagatttattcagtggcaatttttcttggtattaatttggccgcatttatcatcatagttttttcctatggaagcatgttttatagtgttcatcaaagtgccataacagcaactgaaatacggaatcaagttaaaaaagagatgatccttgccaaacgttttttctttatagtatttactgatgcattatgctggatacccatttttgtagtgaaatttctttcactgcttcaggtagaaataccaggtaccataacctcttgggtagtgatttttattctgcccattaacagtgctttgaacccaattctctatactctgaccacaagaccatttaaagaaatgattcatcggttttggtataactacagacaaagaaaatctatggacagcaaaggtcagaaaacatatgctccatcattcatctgggtggaaatgtggccactccaggagatgccacctgagttaatgaagccggaccttttcacatacccctgtgaaatgtcactgatttctcaatcaacgagactcaattcctattcatgactcgag

SEQ ID NO: 9 - protein, 185 aa, Homo sapiens
MPRLFLFHLLEFCLLLNQFSRAVAAKWKDDVIKLCGRELVRAQIAICGMSTWSKRSLSQEDAPQTPRPVAEIVPSFINKDTETIIIMLEFIANLPPELKAALSERQPSLPELQQYVPALKDSNLSFEEFKKLIRNRQSEAADSNPSELKYLGLDTHSQKKRRPYVALFEKCCLIGCTKRSLAKYC

SEQ ID NO: 10 - protein, 29 aa, Artificial
  Serelaxin heavy chain
DSWMEEVIKLCGRELVRAQIAICGMSTWS

SEQ ID NO: 11 - protein, 24 aa, Artificial
  Serelaxin light chain
QLYSALANKCCHVGCTKRSLARFC

SEQ ID NO: 12 - protein, 18 aa, Artificial
  short serelaxin heavy chain
VIKLCGRELVRAQIAICG

SEQ ID NO: 13 - protein, 21 aa, Artificial
  short serelaxin light chain
SALANKCCHVGCTKRSLARFC

SEQ ID NO: 14 - DNA, 20 bp, Artificial
  ANP Forward primer
tgccggtagaagatgaggtc

SEQ ID NO: 15 - DNA, 20 bp, Artificial
  ANP Reverse Primer
tgcttttcaagagggcagat

SEQ ID NO: 16 - DNA, 24 bp, Artificial
  beta-MHC Forward primer
gccaacaccaacctgtccaagttc

SEQ ID NO: 17 - DNA, 24 bp, Artificial
  beta-MHC Reverse primer
tgcaaaggctccaggtctgagggc

SEQ ID NO: 18 - DNA, 20 bp, Artificial
  BNP Forward primer
ctgaaggtgctgtcccagat

SEQ ID NO: 19 - DNA, 20 bp, Artificial
  BNP Reverse primer
ccttggtccttcaagagctg

SEQ ID NO: 20 - DNA, 20 bp, Artificial
  Col1a1 Forward primer
gtgttccctactcagccgtc

SEQ ID NO: 21 - DNA, 20 bp, Artificial
  Col1a1 Reverse Primer
actcgaacgggaatccatcg

SEQ ID NO: 22 - DNA, 20 bp, Artificial
  Col3a1 Forward primer
tgactgtcccacgtaagcac

SEQ ID NO: 23 - DNA, 20 bp, Artificial
  Col3a1 Reverse primer
gagggccatagctgaactga

SEQ ID NO: 24 - DNA, 24 bp, Artificial
  Hprt1 Forward primer
gaggagtcctgttgatgttgccag

SEQ ID NO: 25 - DNA, 24 bp, Artificial
  Hprt1 Reverse primer
ggctggcctataggctcatagtgc

SEQ ID NO: 26 - DNA, 21 bp, Artificial
  Postn Forward primer
acaaaagggttcaagggccta

SEQ ID NO: 27 - DNA, 20 bp, Artificial
  Postn Reverse primer
ttggcttctgttggttgtca

SEQ ID NO: 28 - DNA, 20 bp, Rattus norvegicus
ccatgcattgtttgtgccga

SEQ ID NO: 29 - DNA, 20 bp, Rattus norvegicus
tttgcaggcacagcttttgg

SEQ ID NO: 30 - DNA, 22 bp, Homo sapiens
ctacaaggacgacgatgacaag

SEQ ID NO: 31 - DNA, 22 bp, Homo sapiens
gaaatagccaagggagcacttg

SEQ ID NO: 32 - DNA, 20 bp, Homo sapiens
ctttcctgggaggtcgttcc

SEQ ID NO: 33 - DNA, 19 bp, Homo sapiens
gttgcgctgctcctgtaac

SEQ ID NO: 34 - DNA, 25 bp, Homo sapiens
ctcatggactaattatggacaggac

SEQ ID NO: 35 - DNA, 25 bp, Homo sapiens
gcaggtcagcaaagaatttatagcc

SEQ ID NO: 36 - DNA, 20 bp, Homo sapiens
ggacctgaaggagctgtcac

SEQ ID NO: 37 - DNA, 24 bp, Homo sapiens
taggctgagagacttgagtttgac

SEQ ID NO: 38 - protein, 142 aa, Homo sapiens
MARYMLLLLLAVWVLTGELWPGAEARAAPYGVRLCGREFIRAVIFTCGGSRWRRSDILAHEAMGDTFPDADADEDSLAGELDEAMGSSEWLALTKSPQAFYRGRPSWQGTPGVLRGSRDVLAGLSSSCCKWGCSKSEISSLC